European Patent Application EP 4 372 010 A1, published May 22, 2024. Title: Novel chimeric receptor composition, recombinant vector, cell, and application thereof. Applicant: 苏州易慕峰医药研究有限公司. Application CN. The sequence listing filed with the application follows.

SEQUENCE LISTING (27 sequences)

SEQ ID NO: 1 - protein, 292 aa, synthetic construct
YFLGRLVPRGRGAAEAATRKQRITETESPYQELQGQRSDVYSDLNTQRPYYKLCARPRRSPAQEDGKVYINMPGRGMGWIRGRRSRHSWEMSEFHNYNLDLKKSDFSTRWQKQRCPVVKSKCRENASPFFFCCFIAVAMGIRFIIMVTIWSAVFLNSLFNQEVQIPLTESYCGPCPKNWICYKNNCYQFFDESKNWYESQASCMSQNASLLKVYSKEDQDLLKLVKSYHWMGLVHIPTNGSWQWEDGSILSPNLLTIIEMQKGDCALYASSFKGYIENCSTPNTYICMQRTV

SEQ ID NO: 2 - protein, 241 aa, synthetic construct
YFLGRLVPRGRGAAEAATRKQRITETESPYQELQGQRSDVYSDLNTQRPYYKLCARPRRSPAQEDGKVYINMPGRGPFFFCCFIAVAMGIRFIIMVTIWSAVFLNSLFNQEVQIPLTESYCGPCPKNWICYKNNCYQFFDESKNWYESQASCMSQNASLLKVYSKEDQDLLKLVKSYHWMGLVHIPTNGSWQWEDGSILSPNLLTIIEMQKGDCALYASSFKGYIENCSTPNTYICMQRTV

SEQ ID NO: 3 - protein, 279 aa, synthetic construct
MIHLGHILFLLLLPVAAAFNQEVQIPLTESYCGPCPKNWICYKNNCYQFFDESKNWYESQASCMSQNASLLKVYSKEDQDLLKLVKSYHWMGLVHIPTNGSWQWEDGSILSPNLLTIIEMQKGDCALYASSFKGYIENCSTPNTYICMQRTVQTTPGERSSLPAFYPGTSGSCSGCGSLSLPLLAGLVAADAVASLLIVGAVFLCARPRRSPAQEDGKVYINMPGRGYFLGRLVPRGRGAAEAATRKQRITETESPYQELQGQRSDVYSDLNTQRPYYK

SEQ ID NO: 4 - protein, 300 aa, synthetic construct
MALPVTALLLPLALLLHAARPFNQEVQIPLTESYCGPCPKNWICYKNNCYQFFDESKNWYESQASCMSQNASLLKVYSKEDQDLLKLVKSYHWMGLVHIPTNGSWQWEDGSILSPNLLTIIEMQKGDCALYASSFKGYIENCSTPNTYICMQRTVTTTPAPRPPTPAPTIASQPLSLRPEACRPAAGGAVHTRGLDFACDIYIWAPLAGTCGVLLLSLVITLYCLCARPRRSPAQEDGKVYINMPGRGYFLGRLVPRGRGAAEAATRKQRITETESPYQELQGQRSDVYSDLNTQRPYYK

SEQ ID NO: 5 - protein, 318 aa, synthetic construct
MALPVTALLLPLALLLHAARPFNQEVQIPLTESYCGPCPKNWICYKNNCYQFFDESKNWYESQASCMSQNASLLKVYSKEDQDLLKLVKSYHWMGLVHIPTNGSWQWEDGSILSPNLLTIIEMQKGDCALYASSFKGYIENCSTPNTYICMQRTVTTTPAPRPPTPAPTIASQPLSLRPEACRPAAGGAVHTRGLDFACDIYIWAPLAGTCGVLLLSLVITLYCKRGRKKLLYIFKQPFMRPVQTTQEEDGCSCRFPEEEEGGCELYFLGRLVPRGRGAAEAATRKQRITETESPYQELQGQRSDVYSDLNTQRPYYK

SEQ ID NO: 6 - protein, 314 aa, synthetic construct
MALPVTALLLPLALLLHAARPFNQEVQIPLTESYCGPCPKNWICYKNNCYQFFDESKNWYESQASCMSQNASLLKVYSKEDQDLLKLVKSYHWMGLVHIPTNGSWQWEDGSILSPNLLTIIEMQKGDCALYASSFKGYIENCSTPNTYICMQRTVIEVMYPPPYLDNEKSNGTIIHVKGKHLCPSPLFPGPSKPFWVLVVVGGVLACYSLLVTVAFIIFWVRSKRSRLLHSDYMNMTPRRPGPTRKHYQPYAPPRDFAAYRSYFLGRLVPRGRGAAEAATRKQRITETESPYQELQGQRSDVYSDLNTQRPYYK

SEQ ID NO: 7 - protein, 314 aa, synthetic construct; identical to SEQ ID NO: 6

SEQ ID NO: 8 - protein, 486 aa, synthetic construct
MALPVTALLLPLALLLHAARPMGWIRGRRSRHSWEMSEFHNYNLDLKKSDFSTRWQKQRCPVVKSKCRENASPFFFCCFIAVAMGIRFIIMVTIWSAVFLNSLFNQEVQIPLTESYCGPCPKNWICYKNNCYQFFDESKNWYESQASCMSQNASLLKVYSKEDQDLLKLVKSYHWMGLVHIPTNGSWQWEDGSILSPNLLTIIEMQKGDCALYASSFKGYIENCSTPNTYICMQRTVGSGEGRGSLLTCGDVEENPGPMGGLEPCSRLLLLPLLLAVSGLRPVQAQAQSDCSCSTVSPGVLAGIVMGDLVLTVLIALAVYFLGRLVPRGRGAAEAATRKQRITETESPYQELQGQRSDVYSDLNTQRPYYKGSGATNFSLLKQAGDVEENPGPMIHLGHILFLLLLPVAAAQTTPGERSSLPAFYPGTSGSCSGCGSLSLPLLAGLVAADAVASLLIVGAVFLCARPRRSPAQEDGKVYINMPGRG

SEQ ID NO: 9 - protein, 22 aa, synthetic construct
GSGATNFSLLKQAGDVEENPGP

SEQ ID NO: 10 - protein, 52 aa, synthetic construct
YFLGRLVPRGRGAAEAATRKQRITETESPYQELQGQRSDVYSDLNTQRPYYK

SEQ ID NO: 11 - protein, 24 aa, synthetic construct
LCARPRRSPAQEDGKVYINMPGRG

SEQ ID NO: 12 - protein, 216 aa, synthetic construct
MGWIRGRRSRHSWEMSEFHNYNLDLKKSDFSTRWQKQRCPVVKSKCRENASPFFFCCFIAVAMGIRFIIMVTIWSAVFLNSLFNQEVQIPLTESYCGPCPKNWICYKNNCYQFFDESKNWYESQASCMSQNASLLKVYSKEDQDLLKLVKSYHWMGLVHIPTNGSWQWEDGSILSPNLLTIIEMQKGDCALYASSFKGYIENCSTPNTYICMQRTV

SEQ ID NO: 13 - protein, 45 aa, synthetic construct
TTTPAPRPPTPAPTIASQPLSLRPEACRPAAGGAVHTRGLDFACD

SEQ ID NO: 14 - protein, 24 aa, synthetic construct
IYIWAPLAGTCGVLLLSLVITLYC

SEQ ID NO: 15 - protein, 93 aa, synthetic construct
MIHLGHILFLLLLPVAAAQTTPGERSSLPAFYPGTSGSCSGCGSLSLPLLAGLVAADAVASLLIVGAVFLCARPRRSPAQEDGKVYINMPGRG

SEQ ID NO: 16 - protein, 113 aa, synthetic construct
MGGLEPCSRLLLLPLLLAVSGLRPVQAQAQSDCSCSTVSPGVLAGIVMGDLVLTVLIALAVYFLGRLVPRGRGAAEAATRKQRITETESPYQELQGQRSDVYSDLNTQRPYYK

SEQ ID NO: 17 - protein, 40 aa, synthetic construct
LRPVQAQAQSDCSCSTVSPGVLAGIVMGDLVLTVLIALAV

SEQ ID NO: 18 - protein, 21 aa, synthetic construct
GSGEGRGSLLTCGDVEENPGP

SEQ ID NO: 19 - protein, 361 aa, synthetic construct
MLLLVTSLLLCELPHPAFLLIPQVQLVESGGGLVQPGGSLRLSCAASGSIFNIPVMGWYRQAPGKQRELVAGISTGGTTNYGDSVKGRFTISRDNAKNTVYLQMNSLKPEDTAVYYCNVLVVSGIGSTLEVWGQGTLVTVSSIEVMYPPPYLDNEKSNGTIIHVKGKHLCPSPLFPGPSKPFWVLVVVGGVLACYSLLVTVAFIIFWVRSKRSRLLHSDYMNMTPRRPGPTRKHYQPYAPPRDFAAYRSRVKFSRSADAPAYQQGQNQLYNELNLGRREEYDVLDKRRGRDPEMGGKPRRKNPQEGLYNELQKDKMAEAYSEIGMKGERRRGKGHDGLYQGLSTATKDTYDALHMQALPPR

SEQ ID NO: 20 - protein, 292 aa, synthetic construct; identical to SEQ ID NO: 1

SEQ ID NO: 21 - protein, 300 aa, synthetic construct; identical to SEQ ID NO: 4

SEQ ID NO: 22 - protein, 318 aa, synthetic construct; identical to SEQ ID NO: 5

SEQ ID NO: 23 - protein, 314 aa, synthetic construct; identical to SEQ ID NO: 6

SEQ ID NO: 24 - protein, 490 aa, synthetic construct
MLLLVTSLLLCELPHPAFLLIPQVQLVQSGAEVKKPGASVKVSCKASGYTFTNYWINWVRQAPGQGLEWIGNIYPSYIYTNYNQEFKDKVTLTVDESTSTAYMELSSLRSEDTAVYYCTRSPYGYDEYGLDYWGQGTTVTVSSGGGGSGGGGSGGGGSDIQLTQSPSSLSASVGDRVTMTCKSSQSLLNTRNQKNYLTWYQQKPGKAPKLLIYWASTRESGVPSRFSGSGSGTDFTLTISSLQPEDFATYYCQNDYVYPLTFGQGTKLEIKIEVMYPPPYLDNEKSNGTIIHVKGKHLCPSPLFPGPSKPFWVLVVVGGVLACYSLLVTVAFIIFWVRSKRSRLLHSDYMNMTPRRPGPTRKHYQPYAPPRDFAAYRSRVKFSRSADAPAYQQGQNQLYNELNLGRREEYDVLDKRRGRDPEMGGKPRRKNPQEGLYNELQKDKMAEAYSEIGMKGERRRGKGHDGLYQGLSTATKDTYDALHMQALPPR

SEQ ID NO: 25 - protein, 812 aa, synthetic construct
MLLLVTSLLLCELPHPAFLLIPQVQLVQSGAEVKKPGASVKVSCKASGYTFTNYWINWVRQAPGQGLEWIGNIYPSYIYTNYNQEFKDKVTLTVDESTSTAYMELSSLRSEDTAVYYCTRSPYGYDEYGLDYWGQGTTVTVSSGGGGSGGGGSGGGGSDIQLTQSPSSLSASVGDRVTMTCKSSQSLLNTRNQKNYLTWYQQKPGKAPKLLIYWASTRESGVPSRFSGSGSGTDFTLTISSLQPEDFATYYCQNDYVYPLTFGQGTKLEIKIEVMYPPPYLDNEKSNGTIIHVKGKHLCPSPLFPGPSKPFWVLVVVGGVLACYSLLVTVAFIIFWVRSKRSRLLHSDYMNMTPRRPGPTRKHYQPYAPPRDFAAYRSRVKFSRSADAPAYQQGQNQLYNELNLGRREEYDVLDKRRGRDPEMGGKPRRKNPQEGLYNELQKDKMAEAYSEIGMKGERRRGKGHDGLYQGLSTATKDTYDALHMQALPPRGSGATNFSLLKQAGDVEENPGPMALPVTALLLPLALLLHAARPFNQEVQIPLTESYCGPCPKNWICYKNNCYQFFDESKNWYESQASCMSQNASLLKVYSKEDQDLLKLVKSYHWMGLVHIPTNGSWQWEDGSILSPNLLTIIEMQKGDCALYASSFKGYIENCSTPNTYICMQRTVTTTPAPRPPTPAPTIASQPLSLRPEACRPAAGGAVHTRGLDFACDIYIWAPLAGTCGVLLLSLVITLYCLCARPRRSPAQEDGKVYINMPGRGYFLGRLVPRGRGAAEAATRKQRITETESPYQELQGQRSDVYSDLNTQRPYYK

SEQ ID NO: 26 - protein, 489 aa, synthetic construct
MLLLVTSLLLCELPHPAFLLIPDIQMTQTTSSLSASLGDRVTISCRASQDISKYLNWYQQKPDGTVKLLIYHTSRLHSGVPSRFSGSGSGTDYSLTISNLEQEDIATYFCQQGNTLPYTFGGGTKLEITGSTSGSGKPGSGEGSTKGEVKLQESGPGLVAPSQSLSVTCTVSGVSLPDYGVSWIRQPPRKGLEWLGVIWGSETTYYNSALKSRLTIIKDNSKSQVFLKMNSLQTDDTAIYYCAKHYYYGGSYAMDYWGQGTSVTVSSAAAIEVMYPPPYLDNEKSNGTIIHVKGKHLCPSPLFPGPSKPFWVLVVVGGVLACYSLLVTVAFIIFWVRSKRSRLLHSDYMNMTPRRPGPTRKHYQPYAPPRDFAAYRSRVKFSRSADAPAYQQGQNQLYNELNLGRREEYDVLDKRRGRDPEMGGKPRRKNPQEGLYNELQKDKMAEAYSEIGMKGERRRGKGHDGLYQGLSTATKDTYDALHMQALPPR

SEQ ID NO: 27 - protein, 811 aa, synthetic construct
MLLLVTSLLLCELPHPAFLLIPDIQMTQTTSSLSASLGDRVTISCRASQDISKYLNWYQQKPDGTVKLLIYHTSRLHSGVPSRFSGSGSGTDYSLTISNLEQEDIATYFCQQGNTLPYTFGGGTKLEITGSTSGSGKPGSGEGSTKGEVKLQESGPGLVAPSQSLSVTCTVSGVSLPDYGVSWIRQPPRKGLEWLGVIWGSETTYYNSALKSRLTIIKDNSKSQVFLKMNSLQTDDTAIYYCAKHYYYGGSYAMDYWGQGTSVTVSSAAAIEVMYPPPYLDNEKSNGTIIHVKGKHLCPSPLFPGPSKPFWVLVVVGGVLACYSLLVTVAFIIFWVRSKRSRLLHSDYMNMTPRRPGPTRKHYQPYAPPRDFAAYRSRVKFSRSADAPAYQQGQNQLYNELNLGRREEYDVLDKRRGRDPEMGGKPRRKNPQEGLYNELQKDKMAEAYSEIGMKGERRRGKGHDGLYQGLSTATKDTYDALHMQALPPRGSGATNFSLLKQAGDVEENPGPMALPVTALLLPLALLLHAARPFNQEVQIPLTESYCGPCPKNWICYKNNCYQFFDESKNWYESQASCMSQNASLLKVYSKEDQDLLKLVKSYHWMGLVHIPTNGSWQWEDGSILSPNLLTIIEMQKGDCALYASSFKGYIENCSTPNTYICMQRTVTTTPAPRPPTPAPTIASQPLSLRPEACRPAAGGAVHTRGLDFACDIYIWAPLAGTCGVLLLSLVITLYCLCARPRRSPAQEDGKVYINMPGRGYFLGRLVPRGRGAAEAATRKQRITETESPYQELQGQRSDVYSDLNTQRPYYK